European Patent Application EP 4 163 354 A2, published April 12, 2023. Title: POLYPEPTIDES HAVING PHOSPHOLIPASE C ACTIVITY AND POLYNUCLEOTIDES ENCODING SAME. Applicant: NOVOZYMES A/S. The sequence listing filed with the application follows.

SEQUENCE LISTING (38 sequences)

SEQ ID NO: 1 - DNA, 969 bp, pseudomonas sp
  source 1..969: mol_type = genomic DNA
atgactcatctcattggtttcgcccctcggttgctggctttttcggcgctgttgctcagccagacggcattcagccaggaaagcccggcattcatcgatcctgcgtcgtggaacaccccgttcaatggcattgcccaggtggcttgtcataactgctacgagaagcaatacgcgaacaccttcagcagtgtgcttgacagtgtacggaccctggagctggacttctgggaccagcgcgatgcggtgagcggcggttcgccccatcactggttcgtgcggcacaaccccggcaccttgttccaatccggcaacgacaataactgcaccggcgatggcaccggcaagaacgacctcgaagcctgtctgaacgacgtcaagaactggagtgacaagcatccggggcacttccccatcacgctgatcctggacaagaaacagggctggtcgaaagaaagttcggggcgcacaccaaaggatttcgacgaactggtggcgcgggtgttccagggcaagctctttaccccccaggatctggcgacgcacattggcagtggcgcgggggccttgcagggcaacctcaagggtaagtcctggcccaccgccaacgatctgcagggcaaggtgctgttggtgctcaaccactcggaaaaccagaagctctcgcagtacgccgaggcccgcacctctaaggctaaggtgttcatttcgccagtaaccaacggccagaacgatatcagtggcaaggtcagcggcatgtccagccagtcatccggctatgtagccatgaacaacatgggcaagggcgacaaaagttgggcaaagcaggcctttgcctacagccatatcggccgcgtctggggtgatgacgaggtgtcgttcgcccagcacatcaaccagaagatcaatctgtcggcgtactacaggttcgccgcgcagagcgctggcggctaccgcatccggccgttctga

SEQ ID NO: 2 - protein, 322 aa, pseudomonas sp
  SIGNAL 1..25
MTHLIGFAPRLLAFSALLLSQTAFSQESPAFIDPASWNTPFNGIAQVACHNCYEKQYANTFSSVLDSVRTLELDFWDQRDAVSGGSPHHWFVRHNPGTLFQSGNDNNCTGDGTGKNDLEACLNDVKNWSDKHPGHFPITLILDKKQGWSKESSGRTPKDFDELVARVFQGKLFTPQDLATHIGSGAGALQGNLKGKSWPTANDLQGKVLLVLNHSENQKLSQYAEARTSKAKVFISPVTNGQNDISGKVSGMSSQSSGYVAMNNMGKGDKSWAKQAFAYSHIGRVWGDDEVSFAQHINQKINLSAYYRFAAQSAGGYRIRPF

SEQ ID NO: 3 - protein, 298 aa, synthetic construct
  REGION 1..298: note = variant
AQESPAFIDPASWNTPFNGIAQVACHNCYEKQYANTFSSVLDSVRTLELDFWDQRDAVSGGSPHHWFVRHNPGTLFQSGNDNNCTGDGTGKNDLEACLNDVKNWSDKHPGHFPITLILDKKQGWSKESSGRTPKDFDELVARVFQGKLFTPQDLATHIGSGAGALQGNLKGKSWPTANDLQGKVLLVLNHSENQKLSQYAEARTSKAKVFISPVTNGQNDISGKVSGMSSQSSGYVAMNNMGKGDKSWAKQAFAYSHIGRVWGDDEVSFAQHINQKINLSAYYRFAAQSAGGYRIRPF

SEQ ID NO: 4 - DNA, 972 bp, pseudomonas chlororaphis
  source 1..972: mol_type = genomic DNA
atgtcccgtctcactcgctttgccctccgtaccgccgtgatgcccctggtgctggccagccagatggcgtccagccaggaggctgtgggattcatttccccggcttcctggtacaccgccttcaacgctatcgcccaggtggcgtgccataactgctacgaaaaacagtacgccggcaccttcaccagcgtgctcgacagcgtgcgcaccctggagctggacttctgggaccaacgcgatgcggtcaccggaggttcgccccgccactggttcgtgcggcacaaccccggcagcctgttccagtccggcaatgacaacaattgcaccggcgacggcaaaggcaccaacgatcttgaggcctgcctcaatgacatcaagctctggagcgacagccatcccgggcacttcccgattaccctgatcctcgacaagaagcagggctggtcgaaggaaagctccgggcgtacgcctaaagacttcgatgacctggtcagccggattttccagggcaagctctacaccccgggcgacctggcccagcacctgggtgtcagcagcagtgccttgcagggctcgctcaagggcaagtcctggccgaccgccagccaactgcagggcaaggtgctgttggtgctcaaccactcggagaaccagaagctctcgcaatacgccgaggcccgcaccaccagcgccaaggtgttcatttccccggtcaccaacggccagaacgatgtcagtggcgaggtcagcggcatgtccaggacgtcgtccggctacgtggccatgaacaacatgggcaagggcgacaagcagtgggccgcgcaagcctttgcctacagccacatcggtcgggtgtggggcgatgacggcgtgtcattcacccagcacatcgccgagaaggtcaatctgtcggcgtattacaaattcgccgaggccaaggatggcaacggctatcgcatccggccgttctga

SEQ ID NO: 5 - protein, 323 aa, pseudomonas chlororaphis
  SIGNAL 1..25
MSRLTRFALRTAVMPLVLASQMASSQEAVGFISPASWYTAFNAIAQVACHNCYEKQYAGTFTSVLDSVRTLELDFWDQRDAVTGGSPRHWFVRHNPGSLFQSGNDNNCTGDGKGTNDLEACLNDIKLWSDSHPGHFPITLILDKKQGWSKESSGRTPKDFDDLVSRIFQGKLYTPGDLAQHLGVSSSALQGSLKGKSWPTASQLQGKVLLVLNHSENQKLSQYAEARTTSAKVFISPVTNGQNDVSGEVSGMSRTSSGYVAMNNMGKGDKQWAAQAFAYSHIGRVWGDDGVSFTQHIAEKVNLSAYYKFAEAKDGNGYRIRPF

SEQ ID NO: 6 - protein, 299 aa, synthetic construct
  REGION 1..299: note = variant
AQEAVGFISPASWYTAFNAIAQVACHNCYEKQYAGTFTSVLDSVRTLELDFWDQRDAVTGGSPRHWFVRHNPGSLFQSGNDNNCTGDGKGTNDLEACLNDIKLWSDSHPGHFPITLILDKKQGWSKESSGRTPKDFDDLVSRIFQGKLYTPGDLAQHLGVSSSALQGSLKGKSWPTASQLQGKVLLVLNHSENQKLSQYAEARTTSAKVFISPVTNGQNDVSGEVSGMSRTSSGYVAMNNMGKGDKQWAAQAFAYSHIGRVWGDDGVSFTQHIAEKVNLSAYYKFAEAKDGNGYRIRPF

SEQ ID NO: 7 - DNA, 972 bp, pseudomonas sp
  source 1..972: mol_type = genomic DNA
atgtcccgtctcactggttttgccctccgtaccgccgtgctgcccctggcactggccagccagatggcgtccagccaggaggccgtgggattcatttccccggcgtcctggtacaccgccttcaacgctatcgcccaggtggcatgccataactgctacgaaaaacagtacgccggcaccttcaccagcgtgctcgatagcgtgcgcaccctggagctggacttctgggaccaacgcgatgcggtcaccggaggttcgccccgccactggttcgtgcggcacaaccccggcagcctgttccagtccggcaatgacaacaattgcaccggcgacggcaacggcaccaacgatctcgaagcctgcctcaacgacatcaagctctggagcgacagccatcccgggcacttcccgattaccctgatcctcgacaagaagcagggctggtcgaaggaaagctccgggcgtacgccgaaagacttcgatgacctggtcagccggattttccagggcaagctctacaccccgggcgacctggcccagcatctgggtgtcagcagcagtgccttgcagggctcgctcaagggcaagtcctggccgaccgccagccaactgcagggcaaggtgctgctggtgctcaaccactcggagaaccagaagctctcgcaatacgccgaggcccgcaccaccagcgccaaggtgttcatttccccggtcaccaacggccagaacgatgtcagtggcgaggtcagcggcatgtcgaggacgtcgtccggctacgtggccatgaacaacatgggcaagggcgacaagcagtgggccgcgcaagcctttgtctacagccacatcggtcgggtgtggggtgatgacggcgtgtcattcacccagcacatcgccgagaaggtcaatctgtcggcgtattacaaattcgccgaggccaaggatggcaacggctatcgcatccgaccgttctga

SEQ ID NO: 8 - protein, 323 aa, pseudomonas sp
  SIGNAL 1..25
MSRLTGFALRTAVLPLALASQMASSQEAVGFISPASWYTAFNAIAQVACHNCYEKQYAGTFTSVLDSVRTLELDFWDQRDAVTGGSPRHWFVRHNPGSLFQSGNDNNCTGDGNGTNDLEACLNDIKLWSDSHPGHFPITLILDKKQGWSKESSGRTPKDFDDLVSRIFQGKLYTPGDLAQHLGVSSSALQGSLKGKSWPTASQLQGKVLLVLNHSENQKLSQYAEARTTSAKVFISPVTNGQNDVSGEVSGMSRTSSGYVAMNNMGKGDKQWAAQAFVYSHIGRVWGDDGVSFTQHIAEKVNLSAYYKFAEAKDGNGYRIRPF

SEQ ID NO: 9 - protein, 299 aa, synthetic construct
  REGION 1..299: note = Variant
AQEAVGFISPASWYTAFNAIAQVACHNCYEKQYAGTFTSVLDSVRTLELDFWDQRDAVTGGSPRHWFVRHNPGSLFQSGNDNNCTGDGNGTNDLEACLNDIKLWSDSHPGHFPITLILDKKQGWSKESSGRTPKDFDDLVSRIFQGKLYTPGDLAQHLGVSSSALQGSLKGKSWPTASQLQGKVLLVLNHSENQKLSQYAEARTTSAKVFISPVTNGQNDVSGEVSGMSRTSSGYVAMNNMGKGDKQWAAQAFVYSHIGRVWGDDGVSFTQHIAEKVNLSAYYKFAEAKDGNGYRIRPF

SEQ ID NO: 10 - DNA, 972 bp, Pseudomonas chlororaphis
  source 1..972: mol_type = genomic DNA
atgtcccgtctcactcgttttgccctccgtacagccgtactgcccctggcgctggccagccagatggcgtccagccaggaggccgcgggattcatttctccggcttcctggtacagcgccttcaacgctatcgcccaggtggcgtgccataactgctacgaaaaacagtacgccagcaccttcaccagtgtgctcgacagcgtgcgtaccctggagctggatttctgggaccagcgcgatgcggtcaccggtggttcggccggtcactggttcgtgcggcacaaccccggcacgctgttccagtccggcaatgacaacaactgcaccggcgacggcaaaggcaccaacgatctcgaggcctgcctcaacgacatcaggctctggagcgacagccatcccgggcacttcccgattaccctgatcctcgacaagaagcagggctggtcgaaggaaagctccgggcgtacgccgaaagacttcgatgatctggtcagccggattttccagggcaagctctataccccgggcgacctggcccagcacctgggtgtcagcagcggtgccttgcagggctcgctcgagggcaagtcctggccgaccgctagccaactgcagggcaaggtgctgctggtgctcaaccactcggagaaccagaagctctcgcaatacgccgaagcccggaccaccagcgccaaggtgttcatttcaccggtcaccaacggccagaacgatgtcagtggcgaggtcagcggcatgtccaggacgtcgtccggttacgtggccatgaacaacatgggcaagggcgacaagcagtgggccgcacaagcctttgcctacagccacatcggtcgggtgtggggtgatgacggcgtgtcattcacccagcacatcgccgagaaggtcaatctgtcggcgtattacaagttcgccgaagccaaggatggcaacggctatcgcatccggccgttctaa

SEQ ID NO: 11 - protein, 323 aa, Pseudomonas chlororaphis
  SIGNAL 1..25
MSRLTRFALRTAVLPLALASQMASSQEAAGFISPASWYSAFNAIAQVACHNCYEKQYASTFTSVLDSVRTLELDFWDQRDAVTGGSAGHWFVRHNPGTLFQSGNDNNCTGDGKGTNDLEACLNDIRLWSDSHPGHFPITLILDKKQGWSKESSGRTPKDFDDLVSRIFQGKLYTPGDLAQHLGVSSGALQGSLEGKSWPTASQLQGKVLLVLNHSENQKLSQYAEARTTSAKVFISPVTNGQNDVSGEVSGMSRTSSGYVAMNNMGKGDKQWAAQAFAYSHIGRVWGDDGVSFTQHIAEKVNLSAYYKFAEAKDGNGYRIRPF

SEQ ID NO: 12 - protein, 296 aa, synthetic construct
  REGION 1..296: note = variant
AAGFISPASWYSAFNAIAQVACHNCYEKQYASTFTSVLDSVRTLELDFWDQRDAVTGGSAGHWFVRHNPGTLFQSGNDNNCTGDGKGTNDLEACLNDIRLWSDSHPGHFPITLILDKKQGWSKESSGRTPKDFDDLVSRIFQGKLYTPGDLAQHLGVSSGALQGSLEGKSWPTASQLQGKVLLVLNHSENQKLSQYAEARTTSAKVFISPVTNGQNDVSGEVSGMSRTSSGYVAMNNMGKGDKQWAAQAFAYSHIGRVWGDDGVSFTQHIAEKVNLSAYYKFAEAKDGNGYRIRPF

SEQ ID NO: 13 - DNA, 969 bp, Pseudomonas protegens
  source 1..969: mol_type = genomic DNA
atgactcatctttcccgtttcgtcccccgcgccctggcgctgtcggcactcttgctcagcccggcggcgttcagccaggaaagcccggcgttcatcgccccggctacctggaataccccgttcaacggcatcgcccaggtggcctgtcacaactgctacgagaagcaatacgcaagcaccttcagcagcgtgctcgacagtgtgcgcaccctggaactggacttctgggaccagcgcgatgcggtgaccggcggctcgccccggcactggttcgtgcggcacaaccccggcaccctgttccagtccggcaacgacaacaattgcacgggcgatggcaccggcaagaacgatctcgaagcctgcctcaacgacgtcaagaactggagcgaaaaccaccccgggcactttcccatcacggtgatcctcgacaagaagcagggctggtcgaaggaaagctcggggcgcacgcccaaggatttcgatgagctggtgacccgggtcttccagggcaagctctataccccccaggacctggccacgcacatcggcagcagcgcgggcgccttgcagggcaacctcaagggcaagtcctggcccaccgccagccagcttcagggcaaggtcctgctggtgctcaaccactcggaaaaccagaagctctcgcagtacgccgaggcccggacttccagcgccaaggtgttcatctcgccggtgaccaatggccagaacgatgtcagcggcaaggtcagtggcatgtccggccagtcgtccggctacgtggccatgaacaacatgtccaagggcgacaagaagtgggcggcccaggcctttgcctacagccatgtgggccgggtctggggcgatgacggggtgtcgttcgcccagcacatcagcgagaaggtcaacctctcggcctactacaagttcgccgagcagaactccggcggctatcgcatccggccgttctga

SEQ ID NO: 14 - protein, 322 aa, Pseudomonas protegens
  SIGNAL 1..25
MTHLSRFVPRALALSALLLSPAAFSQESPAFIAPATWNTPFNGIAQVACHNCYEKQYASTFSSVLDSVRTLELDFWDQRDAVTGGSPRHWFVRHNPGTLFQSGNDNNCTGDGTGKNDLEACLNDVKNWSENHPGHFPITVILDKKQGWSKESSGRTPKDFDELVTRVFQGKLYTPQDLATHIGSSAGALQGNLKGKSWPTASQLQGKVLLVLNHSENQKLSQYAEARTSSAKVFISPVTNGQNDVSGKVSGMSGQSSGYVAMNNMSKGDKKWAAQAFAYSHVGRVWGDDGVSFAQHISEKVNLSAYYKFAEQNSGGYRIRPF

SEQ ID NO: 15 - protein, 298 aa, synthetic construct
  REGION 1..298: note = variant
AQESPAFIAPATWNTPFNGIAQVACHNCYEKQYASTFSSVLDSVRTLELDFWDQRDAVTGGSPRHWFVRHNPGTLFQSGNDNNCTGDGTGKNDLEACLNDVKNWSENHPGHFPITVILDKKQGWSKESSGRTPKDFDELVTRVFQGKLYTPQDLATHIGSSAGALQGNLKGKSWPTASQLQGKVLLVLNHSENQKLSQYAEARTSSAKVFISPVTNGQNDVSGKVSGMSGQSSGYVAMNNMSKGDKKWAAQAFAYSHVGRVWGDDGVSFAQHISEKVNLSAYYKFAEQNSGGYRIRPF

SEQ ID NO: 16 - DNA, 969 bp, Pseudomonas protegens
  source 1..969: mol_type = genomic DNA
atgactcatctttcccgtttcgtcccccgcgccctggcgctgtcggcactcctgctcagcccggcggcgttcagccaggaaagcccggcgttcatcgccccggctacctggaataccccgttcaacggcatcgcccaggtggcctgtcacaactgctacgagaagcagtacgcaagcacctttagcagcgtgctcgacagtgtgcgcaccctggaactggacttctgggaccagcgcgatgcggtgaccggcggctcgccccggcactggttcgtgcggcacaaccccggcaccctgttccagtccggcaacgacaacaattgcacgggcgatggcaccggcaagaacgatctcgaagcctgcctcaacgacgtgaagaactggagcgacaaccaccccgggcactttcccattacggtgatcctcgacaagaagcagggctggtcgaaggaaagctcggggcgcacgcccaaggatttcgatgagctggtgacccgggtcttccagggcaagctctataccccccaggacctggccacgcacatcggcagcagcgcgggcgccttgcagggcaacctcaagggcaagtcctggcccaccgccagccagcttcagggcaaggtcctgctggtgctcaaccactcggaaaaccagaagctctcgcagtacgccgaggcccggacttccagcgccaaggtgttcatctcgccggtgaccaatggccagaacgatgtcagtggcaaggtcagtggcatgtccggccagtcgtccggctacgtggccatgaacaacatgtccaagggcgacaagaagtgggcggcccaggcctttgcctacagccatgtgggccgggtctggggcgatgacggggtgtcgttcgcccagcacatcagcgagaaggtcaacctctcggcctactacaagttcgccgagcagaacgccggcggctatcgcatccggccgttctga

SEQ ID NO: 17 - protein, 322 aa, Pseudomonas protegens
  SIGNAL 1..25
MTHLSRFVPRALALSALLLSPAAFSQESPAFIAPATWNTPFNGIAQVACHNCYEKQYASTFSSVLDSVRTLELDFWDQRDAVTGGSPRHWFVRHNPGTLFQSGNDNNCTGDGTGKNDLEACLNDVKNWSDNHPGHFPITVILDKKQGWSKESSGRTPKDFDELVTRVFQGKLYTPQDLATHIGSSAGALQGNLKGKSWPTASQLQGKVLLVLNHSENQKLSQYAEARTSSAKVFISPVTNGQNDVSGKVSGMSGQSSGYVAMNNMSKGDKKWAAQAFAYSHVGRVWGDDGVSFAQHISEKVNLSAYYKFAEQNAGGYRIRPF

SEQ ID NO: 18 - DNA, 837 bp, Bacillus sp
  source 1..837: mol_type = genomic DNA
atgaaacatcatcgttttcgaacgaatttattatcggctctttcagtaagttcaattgtcatcacctcaatcatcggctccactcaaaccacgtacgcttggtcggccgatgctccgcatgatcccaatcagagcacacacctgtttatcgtgaacggtgctgtcaatctggttgccaacaatacggacccgcagatcaacaagcccaccgcgctgttgcaacagtggcgttctcaatgggagcaagggttgtacgatgccgatcatctgaacccttactatgactccggcacttttatgtcccatttttacgatccggacacgcaaacgaactacgcagggttgtcgtacccgacagcacgccaaacaggggcaaaatattttacgattgcctcgaatgactatcaagcaggggatatgtcggatgcattttacaatttaggcttgtccctgcactatttcacagatgtcacgatgccgcttcatgccggaaatatttccaatctcgatcacgaagcacccggctaccatgcgaaactcgaagcgtatgccgaatcgattcaaaatcaagtgacgcctccgactgccggactctacaattgggtctctccgaatgatccggaactctggattcatcaagcggctgtgcaagcgaaatccgtcttgccgcaagtatggaacagtgatatcacgagttggttctgggaggcggctttcagcaattactactcgcaacaatggcacaacgcagtaaccactccggtcctgaatcagttgtcgcaagcggaggcagagaccgccggatatattgatctgttcttccgtgtaaacggttag

SEQ ID NO: 19 - protein, 278 aa, Bacillus sp
  SIGNAL 1..33
MKHHRFRTNLLSALSVSSIVITSIIGSTQTTYAWSADAPHDPNQSTHLFIVNGAVNLVANNTDPQINKPTALLQQWRSQWEQGLYDADHLNPYYDSGTFMSHFYDPDTQTNYAGLSYPTARQTGAKYFTIASNDYQAGDMSDAFYNLGLSLHYFTDVTMPLHAGNISNLDHEAPGYHAKLEAYAESIQNQVTPPTAGLYNWVSPNDPELWIHQAAVQAKSVLPQVWNSDITSWFWEAAFSNYYSQQWHNAVTTPVLNQLSQAEAETAGYIDLFFRVNG

SEQ ID NO: 20 - protein, 246 aa, synthetic construct
  REGION 1..246: note = variant
AWSADAPHDPNQSTHLFIVNGAVNLVANNTDPQINKPTALLQQWRSQWEQGLYDADHLNPYYDSGTFMSHFYDPDTQTNYAGLSYPTARQTGAKYFTIASNDYQAGDMSDAFYNLGLSLHYFTDVTMPLHAGNISNLDHEAPGYHAKLEAYAESIQNQVTPPTAGLYNWVSPNDPELWIHQAAVQAKSVLPQVWNSDITSWFWEAAFSNYYSQQWHNAVTTPVLNQLSQAEAETAGYIDLFFRVNG

SEQ ID NO: 21 - DNA, 852 bp, Bacillus thuringiensis
  source 1..852: mol_type = genomic DNA
atgaaaaagaaagtacttgctttagcagcagctattacattagtagctcctttacaaagcgttgcatttgctcatgaaaatgatgggggaagtaaaataaaaatagttcaccgctggtctgctgaagataaacataaagaaggcgtaaattctcatttatggattgtaaaccgtgcgattgatattatgtctcgcaatacaacacttgtaaaacaagatcgagttgcacaattaaatgaatggcgtacagagttagagaacggtatttatgctgctgactatgaaaatccttattatgataatagcacatttgcttcacatttctatgatccagacaatggaaaaacatatattccatttgcaaagcaggcaaaagaaactggagctaaatattttaaattagcgggtgaatcatacaaaaataaagatatgaaacaagcattcttctatttaggattatctcttcattatttaggagatgtaaatcaaccgatgcatgcggcaaactttacaaatctttcgtatccacaaggattccattctaaatatgaaaactttgtagatacgataaaagataattataaagtaacggatggaaatggatattggaattggaaaggtacaaatccagaagattggatccatggagcggcagtagtggcgaaacaagattactctggaattgtaaatgataatacgaaagattggttcgtaaaagcagctgtgtcacaagaatatgcagataaatggcgtgctgaagttacaccgatgacaggtaagcgattaatggatgcacaacgtgttactgctggatacattcagctttggtttgatacgtacggagatcgttaa

SEQ ID NO: 22 - protein, 283 aa, Bacillus thuringiensis
  SIGNAL 1..24
  PROPEP 25..38
MKKKVLALAAAITLVAPLQSVAFAHENDGGSKIKIVHRWSAEDKHKEGVNSHLWIVNRAIDIMSRNTTLVKQDRVAQLNEWRTELENGIYAADYENPYYDNSTFASHFYDPDNGKTYIPFAKQAKETGAKYFKLAGESYKNKDMKQAFFYLGLSLHYLGDVNQPMHAANFTNLSYPQGFHSKYENFVDTIKDNYKVTDGNGYWNWKGTNPEDWIHGAAVVAKQDYSGIVNDNTKDWFVKAAVSQEYADKWRAEVTPMTGKRLMDAQRVTAGYIQLWFDTYGDR

SEQ ID NO: 23 - DNA, 852 bp, Bacillus pseudomycoides
  source 1..852: mol_type = genomic DNA
atgaaaaagaaagtattagccttagcagcagctattacattagtagcaccattgcaaagtgtagcgtttgcccatgaaaatgagggcggaaataaggtaagagtaattcaatattggtctgctgaagataaacatgcagaaggtgtaaactcccatttatggattgtcaatcgtgcaattgatattatgtctcgtaatacaacggttgtaaaacaagatcaagttgcagtattaaatgaatggcgtacagagttagagaatggtatatatgctgctgattatgaaaacccttactatgataacagtacatttgcttctcatttctacgagcctgatacagggaagacatatataccttttgctaagcaggcaaaagaaactggggctaaatattttaaacttgctggtgaagcttatcaaaagcaagatatgaaacaagcattcttctatttgggtttatcccttcattacttaggcgatgtcaatcaaccgatgcatgcagcaaactttacaaatctttcttatccacaaggtttccactccaaatatgaaaattttgtagatacaataaaaaataattataaagtggctgatggaaatggatattggaattggaaaggagtaaatcctgaagactggattcatggagcggctgtagctgctaagcaagattatgctggtattgtaaatggcactacaaaagattggttcgtaagagcggcagtttcacaagaatatgcagataaatggcgtgcagaagttacactaacaacaggaaaacgtttagtagaagcacagcgtgtcacagcgggatatattcagctttggtttgatacgtatgtaaatcgctag

SEQ ID NO: 24 - protein, 283 aa, Bacillus pseudomycoides
  SIGNAL 1..24
  PROPEP 25..38
MKKKVLALAAAITLVAPLQSVAFAHENEGGNKVRVIQYWSAEDKHAEGVNSHLWIVNRAIDIMSRNTTVVKQDQVAVLNEWRTELENGIYAADYENPYYDNSTFASHFYEPDTGKTYIPFAKQAKETGAKYFKLAGEAYQKQDMKQAFFYLGLSLHYLGDVNQPMHAANFTNLSYPQGFHSKYENFVDTIKNNYKVADGNGYWNWKGVNPEDWIHGAAVAAKQDYAGIVNGTTKDWFVRAAVSQEYADKWRAEVTLTTGKRLVEAQRVTAGYIQLWFDTYVNR

SEQ ID NO: 25 - protein, 260 aa, synthetic construct
  REGION 1..260: note = variant
AHENEGGNKVRVIQYWSAEDKHAEGVNSHLWIVNRAIDIMSRNTTVVKQDQVAVLNEWRTELENGIYAADYENPYYDNSTFASHFYEPDTGKTYIPFAKQAKETGAKYFKLAGEAYQKQDMKQAFFYLGLSLHYLGDVNQPMHAANFTNLSYPQGFHSKYENFVDTIKNNYKVADGNGYWNWKGVNPEDWIHGAAVAAKQDYAGIVNGTTKDWFVRAAVSQEYADKWRAEVTLTTGKRLVEAQRVTAGYIQLWFDTYVNR

SEQ ID NO: 26 - DNA, 852 bp, Bacillus mycoides
  source 1..852: mol_type = genomic DNA
atgaaaaagaaagtattagccttagcagcagctattacattagtagcaccattgcaaagtgtagcgtttgcccatgaaaatgagggcggaaataaggtaagagtaattcaatattggtctgctgaagataaacatgcagaaggtgtaaactcccatttatggattgtcaatcgtgcaattgatattatgtctcgtaatacaacggttgtaaaacaagatcaagttgcattattaaatgaatggcgtacagagttagagaatggtatatatgctgctgattatgaaaacccttattatgataacagtacatttgcttctcatttctacgatcctgacacagggaagacatatataccttttgctaagcaggcaaaagaaactggggctaaatattttaaacttgctggtgaagcctatcaaaagcaagaaataaaacaagcattcttctatttaggcttatcgcttcattacttaggagatgtaaatcaaccaatgcatgcagcaaactttacaaatctttcttatccacaaggtttccactccaaatatgaaaattttgtagatacaataaaaaataattataaagtggctgatggaaatggatattggaattggaaaggagtaaatcctgaagactggattcatggagcggctgtagctgctaagcaagattatgctggtattgtaaatggcactacaaaagattggttcgtaagagcggcagtttcacaagaatatgcagataaatggcgtgcagaagttacactaacaacaggaaaacgtttagtagaagcacagcgtgtcacagcgggatatattcagctttggtttgatacatatgtaaatcgctag

SEQ ID NO: 27 - protein, 283 aa, Bacillus mycoides
  SIGNAL 1..24
  PROPEP 25..38
MKKKVLALAAAITLVAPLQSVAFAHENEGGNKVRVIQYWSAEDKHAEGVNSHLWIVNRAIDIMSRNTTVVKQDQVALLNEWRTELENGIYAADYENPYYDNSTFASHFYDPDTGKTYIPFAKQAKETGAKYFKLAGEAYQKQEIKQAFFYLGLSLHYLGDVNQPMHAANFTNLSYPQGFHSKYENFVDTIKNNYKVADGNGYWNWKGVNPEDWIHGAAVAAKQDYAGIVNGTTKDWFVRAAVSQEYADKWRAEVTLTTGKRLVEAQRVTAGYIQLWFDTYVNR

SEQ ID NO: 28 - DNA, 870 bp, Listeria innocua
  source 1..870: mol_type = genomic DNA
atgaaattcaaaaaggtagttctaggtatgtgtttgactgcaagtgttctagtctttccggtaacgataaaagcaagtgcctgttgcgatgaatatttacaagcacccgcagctccgcatgatatcgacagtaaattaccacataaacttagttggtccgcggataacccgacaaatactgacgtaaatacacactattggctttttaaacaagctgaaaaaatactagctaaagatgtaaatcatatacgagctaatttaatgaatgagcttaaaaatttcgataaacaaattgctcaaggtatatatgatgcggatcataaaaatccatattatgatactagtacatttttatctcatttttataatcctgatagagataatacttatttgccgggttttgctaatgcgaaaataactggagccaagtatttcaatcaatcggtggctgattatcgagaaggtaaatttgacacagcattttataaattaggtctagcaatccattattatacggatattagtcaacctatgcacgccaataattttaccgcaatatcatacccaccaggctaccactgcgcatatgaaaattatgtggatactattaaacacaattatcaagcaacagaagacatggtagtgaaaagattttgctcagatgacgtgaaagtctggctctatgaaaatgcgaaaagagcaaaagccgactaccctaaaatagtcaatgcaaaaactaaaaaatcatatttagtaggaaattccaaatggaaaaaggatacagtggaacctactggagctagactaagagattcacagcaaactttggcaggctttttagaattttggtccaaaaaaacaaatgaataa

SEQ ID NO: 29 - protein, 289 aa, Listeria innocua
  SIGNAL 1..27
  PROPEP 28..51
MKFKKVVLGMCLTASVLVFPVTIKASACCDEYLQAPAAPHDIDSKLPHKLSWSADNPTNTDVNTHYWLFKQAEKILAKDVNHIRANLMNELKNFDKQIAQGIYDADHKNPYYDTSTFLSHFYNPDRDNTYLPGFANAKITGAKYFNQSVADYREGKFDTAFYKLGLAIHYYTDISQPMHANNFTAISYPPGYHCAYENYVDTIKHNYQATEDMVVKRFCSDDVKVWLYENAKRAKADYPKIVNAKTKKSYLVGNSKWKKDTVEPTGARLRDSQQTLAGFLEFWSKKTNE

SEQ ID NO: 30 - protein, 263 aa, synthetic construct
  REGION 1..263: note = variant
  PROPEP 1..25
ACCDEYLQAPAAPHDIDSKLPHKLSWSADNPTNTDVNTHYWLFKQAEKILAKDVNHIRANLMNELKNFDKQIAQGIYDADHKNPYYDTSTFLSHFYNPDRDNTYLPGFANAKITGAKYFNQSVADYREGKFDTAFYKLGLAIHYYTDISQPMHANNFTAISYPPGYHCAYENYVDTIKHNYQATEDMVVKRFCSDDVKVWLYENAKRAKADYPKIVNAKTKKSYLVGNSKWKKDTVEPTGARLRDSQQTLAGFLEFWSKKTNE

SEQ ID NO: 31 - DNA, 849 bp, synthetic construct
  misc_feature 1..849: note = variant
  source 1..849: mol_type = other DNA
atgaaaaagaaagtattagcactagcagctatggttgctttagctgcgccagttcaaagtgtagtatttgcacaaacaaataatagtgaaagtcctgcaccgattttaagatggtcagctgaggataagcataatgaggggattaactctcatttgtggattgtaaatcgtgcaattgacatcatgtctcgtaatacaacgattgtgaatccgaatgaaactgcattattaaatgagtggcgtgctgatttagaaaatggtatttattctgctgattacgagaatccttattatgatgatagtacatatgcttctcacttttatgatccggatactggaacaacatatattccttttgcgaaacatgcaaaagaaacaggcgcaaaatattttaaccttgctggtcaagcataccaaaatcaagatatgcagcaagcattcttctacttaggattatcgcttcattatttaggagatgtgaatcagccaatgcatgcagcatcttttacggatctttcttatccaatgggtttccattctaaatacgaaaattttgttgatacaataaaaaataactatattgtttcagatagcaatggatattggaattggaaaggagcaaacccagaagattggattgaaggagcagcggtagcagctaaacaagattatcctggcgttgtgaacgatacgacaaaagattggtttgtaaaagcagccgtatctcaagaatatgcagataaatggcgtgcggaagtaacaccggtgacaggaaagcgtttaatggaagcgcagcgcgttacagctggttatattcatttgtggtttgatacgtatgtaaatcgctaa

SEQ ID NO: 32 - protein, 282 aa, synthetic construct
  REGION 1..282: note = variant
  SIGNAL 1..20
  PROPEP 21..37
MKKKVLALAAMVALAAPVQSVVFAQTNNSESPAPILRWSAEDKHNEGINSHLWIVNRAIDIMSRNTTIVNPNETALLNEWRADLENGIYSADYENPYYDDSTYASHFYDPDTGTTYIPFAKHAKETGAKYFNLAGQAYQNQDMQQAFFYLGLSLHYLGDVNQPMHAASFTDLSYPMGFHSKYENFVDTIKNNYIVSDSNGYWNWKGANPEDWIEGAAVAAKQDYPGVVNDTTKDWFVKAAVSQEYADKWRAEVTPVTGKRLMEAQRVTAGYIHLWFDTYVNR

SEQ ID NO: 33 - protein, 27 aa, synthetic construct
  REGION 1..27: note = signal peptide
MKKPLGKIVASTALLISVAFSSSIASA

SEQ ID NO: 34 - DNA, 1020 bp, Amycolatopsis azurea
  source 1..1020: mol_type = genomic DNA
atgaaactcgtccccgcggtatccctcgtcggcgtgatcttggcggcttcgctgtccggaacggtcgcgaacgccgacgccgccaaggtctcccacgtgacaacggtcggcgtccacaacacctacgagaccggtgcctacgactacctggcgcgctcgctggacgccggtacctcgctgatcgaactcgacgtctggccgaacatcatcactcgcgagtggaaagtgagtcactcgaacccgttggggaacaacaacaactgcgtcgcggcgagtacgccgtcgcagttgtactccggtgggcggaacaagaacctcgaacactgcctcgatgacatccgcgtctggctgggcgcgcatccggacagcaaaccggtcacgctcaaactggagatgaagaccgggttcgccgacaaccgcggcctcggcccggacgaactcgacgcgtccatccgggcacatctgggcagtacggtgttccggccggcggacctgctcggcgggtacgcgacgctcgacgacgcggccaaagcggacaactggccgtccctggacgcgctgcggggcaaggtgatcatcgagatcatccccggcacggtcgaagagggaaatccgacggacacgctcaagaccgacgtcgagtacgggcgatatctgcggtcgctcaaggacgcgggccgcgtcggcgaggtgcagatcttcccgacggtgcacggcgcggcacccggcgacccgcgcacgaagtacgccgacgccgggctgcggccgtggttcgtggtcttcgacggcgacgccaccgcgttcctgacgcagaccgggcccggctggtacgacgacaaccactactacgtggtgatgaccgacgcgcacaacgtcgcgccggccatcgactcccgtgcccccacggtggaccaggcgagcgcgcgagcggccctgctggcgaagaaccacgcttcggtgctgacctcggattggacggggctgaccaccgtgctgccgcaggtacttccgcgcggctag

SEQ ID NO: 35 - protein, 339 aa, Amycolatopsis azurea
  SIGNAL 1..27
MKLVPAVSLVGVILAASLSGTVANADAAKVSHVTTVGVHNTYETGAYDYLARSLDAGTSLIELDVWPNIITREWKVSHSNPLGNNNNCVAASTPSQLYSGGRNKNLEHCLDDIRVWLGAHPDSKPVTLKLEMKTGFADNRGLGPDELDASIRAHLGSTVFRPADLLGGYATLDDAAKADNWPSLDALRGKVIIEIIPGTVEEGNPTDTLKTDVEYGRYLRSLKDAGRVGEVQIFPTVHGAAPGDPRTKYADAGLRPWFVVFDGDATAFLTQTGPGWYDDNHYYVVMTDAHNVAPAIDSRAPTVDQASARAALLAKNHASVLTSDWTGLTTVLPQVLPRG

SEQ ID NO: 36 - protein, 313 aa, synthetic construct
  REGION 1..313: note = Mature polypeptide with extra N term. alanine
AAKVSHVTTVGVHNTYETGAYDYLARSLDAGTSLIELDVWPNIITREWKVSHSNPLGNNNNCVAASTPSQLYSGGRNKNLEHCLDDIRVWLGAHPDSKPVTLKLEMKTGFADNRGLGPDELDASIRAHLGSTVFRPADLLGGYATLDDAAKADNWPSLDALRGKVIIEIIPGTVEEGNPTDTLKTDVEYGRYLRSLKDAGRVGEVQIFPTVHGAAPGDPRTKYADAGLRPWFVVFDGDATAFLTQTGPGWYDDNHYYVVMTDAHNVAPAIDSRAPTVDQASARAALLAKNHASVLTSDWTGLTTVLPQVLPRG

SEQ ID NO: 37 - DNA, 771 bp, synthetic construct
  misc_feature 1..771: note = Synthetic gene
  source 1..771: mol_type = other DNA
gaagatgacgcacaaccgcctattacagcaaaatggtcagcggaagatccgcatcatgaagatacaaatacacatctgtggattgttcgccatgccatggagattatggcgaataacaaagatgttgtcaaacctggcgaagtcgaacaactgaaacaatggcaatcagatctggaacagggcatttatgatgcagatcatgcaaacccgtattatgataatgcaacatttgcgagccatttttatgatccggatacaggcaaatcatatattccgctggcagcacatgcaaaaacaacaagcgttaaatactttaaaagagcaggcgaagcgtatcagaaaggcgatcataaacaagcgttttacaatctgggcctggcgctgcattatattggcgatctgaatcaaccgatgcatgcagcgaattttacaaatctgtcatatccgcaaggctttcatagcaaatatgaaaactatgtcgatagctttaaagaagattacgcggtcaaagatggcgaaggctattggcattggaaaggcacaaatccggaagattggctgcatggcacagcagttgcagcaaaaaaagattatccggatatcgtcaacgatacaacgaaagcatggtttgttaaagcagcagtctcaaatagctatgcagcaaaatggcgtgcagcagttgttccggcaacaggcaaaagactgacagaagcacaaagaattctggcaggctatatgcaactgtggtttgatacatatgtcaacaaataa

SEQ ID NO: 38 - protein, 280 aa, Bacillus macauensis
  REGION 1..24: note = signal peptide
  PROPEP 25..35
MKKTFVAVATAALLVTGFQGNASAEDDAQPPITAKWSAEDPHHEDTNTHLWIVRHAMEIMANNKDVVKPGEVEQLKQWQSDLEQGIYDADHANPYYDNATFASHFYDPDTGKSYIPLAAHAKTTSVKYFKRAGEAYQKGDHKQAFYNLGLALHYIGDLNQPMHAANFTNLSYPQGFHSKYENYVDSFKEDYAVKDGEGYWHWKGTNPEDWLHGTAVAAKKDYPDIVNDTTKAWFVKAAVSNSYAAKWRAAVVPATGKRLTEAQRILAGYMQLWFDTYVNK